European Patent Application EP 4 148 136 A1, published March 15, 2023. Title: AN ENGINEERED YEAST CELL FOR THE DELIVERY OF ANTIBIOTIC-INACTIVATING ENZYMES. Applicant: DA VOLTERRA. The sequence listing filed with the application follows.

SEQUENCE LISTING (114 sequences)

SEQ ID NO: 1 - DNA, 116 bp, ARTIFICIAL
  intron of the PRE3 gene
gtatgtatataagaatttttcctcccactttattgtttctaaaagttcaatgaagtaaagtctcaattggccttattactaactaataggtatcttataatcacctaataaaatag

SEQ ID NO: 2 - DNA, 419 bp, artificial
  TEF1 promoter sequence
cacacaccatagcttcaaaatgtttctactccttttttactcttccagattttctcggactccgcgcatcgccgtaccacttcaaaacacccaagcacagcatactaaatttcccctctttcttcctctagggtgtcgttaattacccgtactaaaggtttggaaaagaaaaaagagaccgcctcgtttctttttcttcgtcgaaaaaggcaataaaaatttttatcacgtttctttttcttgaaaatttttttttttgatttttttctctttcgatgacctcccattgatatttaagttaataaacggtcttcaatttctcaagtttcagtttcatttttcttgttctattacaactttttttacttcttgctcattagaaagaaagcatagcaatctaatctaagttttaattacaa

SEQ ID NO: 3 - DNA, 166 bp, artificial
  ADH1 terminator sequence
gcgaatttcttatgatttatgatttttattattaaataagttataaaaaaaataagtgtatacaaattttaaagtgactcttaggttttaaaacgaaaattcttattcttgagtaactctttcctgtaggtcaggttgctttctcaggtatagcatgaggtcgctc

SEQ ID NO: 4 - DNA, 267 bp, artificial
  alpha-factor signal
atgagatttccttcaatttttactgctgttttattcgcagcatcctccgcattagctgctccagtcaacactacaacagaagatgaaacggcacaaattccggctgaagctgtcatcggttactcagatttagaaggggatttcgatgttgctgttttgccattttccaacagcacaaataacgggttattgtttataaatactactattgccagcattgctgctaaagaagaaggggtatctctcgagaaaagagaggctgaagct

SEQ ID NO: 5 - protein, 89 aa, artificial
  alpha-factor signal
MRFPSIFTAVLFAASSALAAPVNTTTEDETAQIPAEAVIGYSDLEGDFDVAVLPFSNSTNNGLLFINTTIASIAAKEEGVSLEKREAEA

SEQ ID NO: 6 - DNA, 57 bp, artificial
  K1 signal peptide of K. lactis
atgaatatattttacatatttttgtttttgctgtcattcgttcaaggtacccgggga

SEQ ID NO: 7 - protein, 19 aa, artificial
  K1 signal peptide of K. lactis
MNIFYIFLFLLSFVQGTRG

SEQ ID NO: 8 - protein, 240 aa, artificial
  VIM 2 WT
VDSSGEYPTVSEIPVGEVRLYQIADGVWSHIATQSFDGAVYPSNGLIVRDGDELLLIDTAWGAKNTAALLAEIEKQIGLPVTRAVSTHFHDDRVGGVDVLRAAGVATYASPSTRRLAEVEGNEIPTHSLEGLSSSGDAVRFGPVELFYPGAAHSTDNLVVYVPSASVLYGGCAIYELSRTSAGNVADADLAEWPTSIERIQQHYPEAQFVIPGHGLPGGLDLLKHTTNVVKAHTNRSVVE

SEQ ID NO: 9 - DNA, 723 bp, artificial
  Nucleic sequence encoding VIM-2 WT
gtagattctagcggtgagtatccgacagtcagcgaaattccggtcggggaggtccggctttaccagattgccgatggtgtttggtcgcatatcgcaacgcagtcgtttgatggcgcagtctacccgtccaatggtctcattgtccgtgatggtgatgagttgcttttgattgatacagcgtggggtgcgaaaaacacagcggcacttctcgcggagattgagaagcaaattggacttcctgtaacgcgtgcagtctccacgcactttcatgacgaccgcgtcggcggcgttgatgtccttcgggcggctggggtggcaacgtacgcatcaccgtcgacacgccggctagccgaggtagaggggaacgagattcccacgcactctctagaaggactctcatcgagcggggacgcagtgcgcttcggtccagtagaactcttctatcctggtgctgcgcattcgaccgacaacttagttgtgtacgtcccgtctgcgagtgtgctctatggtggttgtgcgatttatgagttgtcacgcacgtctgcggggaacgtggccgatgccgatctggctgaatggcccacctccattgagcggattcaacaacactacccggaagcacagttcgtcattccggggcacggcctgccgggcggtctagacttgctcaagcacacaacgaatgttgtaaaagcgcacacaaatcgctcagtcgttgagtag

SEQ ID NO: 10 - protein, 235 aa, artificial
  VIM-2 [V1M V10A Q34R E130D Q22H DCT236]
MDSSGEYPTASEIPVGEVRLYHIADGVWSHIATRSFDGAVYPSNGLIVRDGDELLLIDTAWGAKNTAALLAEIEKQIGLPVTRAVSTHFHDDRVGGVDVLRAAGVATYASPSTRRLAEVEGNEIPTHSLDGLSSSGDAVRFGPVELFYPGAAHSTDNLVVYVPSASVLYGGCAIYELSRTSAGNVADADLAEWPTSIERIQQHYPEAQFVIPGHGLPGGLDLLKHTTNVVKAHTN

SEQ ID NO: 11 - DNA, 708 bp, artificial
  nucleic sequence encoding VIM-2 [V10A Q34R E130D Q22H DCT236]
atggattctagcggtgagtatccgacagccagcgaaattccggtcggggaagtccggctttaccatattgccgatggagtttggtcgcatatcgcaacgcggtcgtttgatggcgcagtctacccgtccaatggtctcattgtccgtgatggtgatgagttgcttttgattgatacagcgtggggtgcgaaaaacacagcggcacttctcgcggagattgagaagcaaattggacttcctgtaacgcgtgcagtctccacgcactttcatgatgaccgcgtcggcggcgttgatgtccttcgggcggctggggtggcaacgtacgcatcaccgtcgacacgccggctagccgaggtagaggggaacgagattcccacgcactctctagatggactctcatcgagcggggacgcagtgcgcttcggtccagtagaactcttctatcctggtgctgcgcattcgaccgacaacttagttgtgtacgtcccgtctgcgagtgtgctctatggtggttgtgcgatttatgagttgtcacgcacgtctgcggggaacgtggccgatgccgatctggctgaatggcccacctccattgagcggattcaacaacactacccggaagcacagttcgtcattccggggcacggcctgccgggcggtctagacttgctcaagcacacaacgaatgttgtaaaagcgcacacaaattaa

SEQ ID NO: 12 - protein, 262 aa, artificial
  P3A protein sequence
MKDDFAKLEEQFDAKLGIFALDTGTNRTVAYRPDERFAFASTIKALTVGVLLQQKSIEDLNQRITYTRDDLVNYNPITEKHVDTGMTLKELADASLRYSDNAAQNLILKQIGGPESLKKELRKIGDEVTNPERFEPELNEVNPGETQDTSTARALVTSLRAFALEDKLPSEKRELLIDWMKRNTTGDALIRAGVPDGWEVADKTGAASYGTRNDIAIIWPPKGDPVVLAVLSSRDKKDAKYDNKLIAEATKVVMKALNMNGK

SEQ ID NO: 13 - protein, 258 aa, artificial
  mature P3A variant (without signal peptide)
  misc_feature (243)..(243): Xaa can be any naturally occurring amino acid
MKDDFAKLEEQFDAKLGIFALDTGTNRTVAYRPDERFAFASTIKALTVGVLLQQKSIEDLNQRITYTRDDLVNYNPITEKHVDTGMTLKELADASLRYSDNAAQNLILKQIGGPESLKKELRKIGDEVTNPERFEPELNEVNPGETQDTSTARALVTSLRAFALEDKLPSEKRELLIDWMKRNTTGDALIRAGVPDGWEVADKTGAASYGTRNDIAIIWPPKGDPVVLAVLSSRDKKDAKYDXKLIAEATKVVMKALN

SEQ ID NO: 14 - protein, 299 aa, artificial
  P3A variant (with signal peptide)
  misc_feature (280)..(280): Xaa can be any naturally occurring amino acid
MIQKRKRTVSFRLVLMCTLLFVSLPITKTSAQASKTEMKDDFAKLEEQFDAKLGIFALDTGTNRTVAYRPDERFAFASTIKALTVGVLLQQKSIEDLNQRITYTRDDLVNYNPITEKHVDTGMTLKELADASLRYSDNAAQNLILKQIGGPESLKKELRKIGDEVTNPERFEPELNEVNPGETQDTSTARALVTSLRAFALEDKLPSEKRELLIDWMKRNTTGDALIRAGVPDGWEVADKTGAASYGTRNDIAIIWPPKGDPVVLAVLSSRDKKDAKYDXKLIAEATKVVMKALNMNGK

SEQ ID NO: 15 - protein, 264 aa, artificial
  P3A  "long version"
TEMKDDFAKLEEQFDAKLGIFALDTGTNRTVAYRPDERFAFASTIKALTVGVLLQQKSIEDLNQRITYTRDDLVNYNPITEKHVDTGMTLKELADASLRYSDNAAQNLILKQIGGPESLKKELRKIGDEVTNPERFEPELNEVNPGETQDTSTARALVTSLRAFALEDKLPSEKRELLIDWMKRNTTGDALIRAGVPDGWEVADKTGAASYGTRNDIAIIWPPKGDPVVLAVLSSRDKKDAKYDNKLIAEATKVVMKALNMNGK

SEQ ID NO: 16 - DNA, 789 bp, artificial
  sequence encoding P3A of seq id 12
atgaaagatgattttgcaaaacttgaggaacaatttgatgcaaaactcggcatctttgcattggataccggtaccaaccggacggtggcgtatcggccggatgagcgttttgcgtttgcgtcgacgattaaagcgttaaccgtgggcgtgcttttgcaacagaaatcaattgaagatctgaaccagcgtattacctatacccgtgatgatcttgtgaactacaacccgattacggaaaaacacgttgatacgggcatgacgctcaaagagcttgcggatgcgtcgcttcgatatagtgacaatgcggcacagaatctcattcttaaacaaattggcggccctgaaagtttgaaaaaagaactgcgtaaaattggtgatgaggttaccaatccggaacgattcgaaccagagttaaatgaagtgaatccgggtgaaacccaggataccagtaccgcacgtgcacttgtcaccagccttcgagcctttgcgcttgaagataaacttccaagtgaaaaacgcgagcttttaatcgattggatgaaacgaaataccaccggcgacgccttaatccgtgccggtgtgccggacggttgggaagtggcggataaaaccggcgcggcaagctatggcacccggaatgacattgccatcatttggccgccaaaaggcgatcctgtcgttcttgcagtgttatccagccgtgataaaaaagacgccaaatatgataataaacttattgcagaggcaaccaaagtggtgatgaaagccttaaacatgaacggcaaataa

SEQ ID NO: 17 - DNA, 774 bp, artificial
  sequence encoding P3A of seq id 14
  misc_feature (727)..(729): n is a, c, g, or t
atgaaagatgattttgcaaaacttgaggaacaatttgatgcaaaactcgggatctttgcattggatacaggtacaaaccggacggtagcgtatcggccggatgagcgttttgcttttgcttcgacgattaaggctttaactgtaggcgtgcttttgcaacagaaatcaatagaagatctgaaccagagaataacatatacacgtgatgatcttgtaaactacaacccgattacggaaaagcacgttgatacgggaatgacgctcaaagagcttgcggatgcttcgcttcgatatagtgacaatgcggcacagaatctcattcttaaacaaattggcggacctgaaagtttgaaaaaggaactgaggaagattggtgatgaggttacaaatcccgaacgattcgaaccagagttaaatgaagtgaatccgggtgaaactcaggataccagtacagcaagagcacttgtcacaagccttcgagcctttgctcttgaagataaacttccaagtgaaaaacgcgagcttttaatcgattggatgaaacgaaataccactggagacgccttaatccgtgccggtgtgccggacggttgggaagtggctgataaaactggagcggcatcatatggaacccggaatgacattgccatcatttggccgccaaaaggagatcctgtcgttcttgcagtattatccagcagggataaaaaggacgccaagtatgatnnnaaacttattgcagaggcaacaaaggtggtaatgaaagccttaaac

SEQ ID NO: 18 - DNA, 795 bp, artificial
  sequence encoding P3A of seq id 15
atgactgagatgaaagatgattttgcgaagctggaagaacagtttgacgcaaaattgggcattttcgcgttggacacgggtacgaatcgtacggttgcctaccgtccggacgagcgcttcgccttcgcgagcacgatcaaagccctgaccgtcggcgtgctgctccagcaaaagagcatcgaggacctgaaccagcgcattacctacacccgtgatgatctggtgaactataatccgatcaccgagaaacacgttgataccggtatgaccctgaaagaactggcagatgcaagcctgcgctacagcgataacgcggctcagaatctgattctgaagcaaatcggtggtccggagagcttgaagaaagaactgcgtaaaatcggcgatgaagtcactaatccggagcgttttgagccggagctgaacgaagtgaatccgggtgaaacgcaagacacgagcaccgcgcgtgcgcttgtcacctccctgcgcgctttcgcactggaagataagctgccgtcggagaaacgcgagctgctgatcgactggatgaagcgcaatacgaccggcgacgcgctgattcgtgcgggcgttccggacggttgggaagtggctgacaagaccggtgcggcgagctacggcacccgtaacgatatcgcgatcatttggccacctaaaggtgacccggtcgtgctggccgtactgagcagccgtgacaagaaagacgcaaagtatgataacaagctgattgcagaggcgaccaaagttgttatgaaggcactgaacatgaatggtaag

SEQ ID NO: 19 - protein, 235 aa, artificial
  VIM-2 variant
MDSSGEYPTVSEIPVGEVRLYQIADGVWSHIATQSFDGAVYPSNGLIVRDGDELLLIDTAWGAKNTAALLAEIEKQIGLPVTRAVSTHFHDDRVGGVDVLRAAGVATYASPSTRRLAEVEGNEIPTHSLEGLSSSGDAVRFGPVELFYPGAAHSTDNLVVYVPSASVLYGGCAIYELSRTSAGNVADADLAEWPTSIERIQQHYPEAQFVIPGHGLPGGLDLLKHTTNVVKAHTN

SEQ ID NO: 20 - protein, 235 aa, artificial
  VIM-2 variant
MDSSGEYPTVSEIPVGEVRLYQIADGVWSHIATRSFDGAVYPSNGLIVRDGDELLLIDTAWGAKNTAALLAEIEKQIGLPVTRAVSTHFHDDRVGGVDVLRAAGVATYASPSTRRLAEVEGNEIPTHSLEGLSSSGDAVRFGPVELFYPGAAHSTDNLVVYVPSASVLYGGCAIYELSRTSAGNVADADLAEWPTSIERIQQHYPEAQFVIPGHGLPGGLDLLKHTTNVVKAHTN

SEQ ID NO: 21 - protein, 235 aa, artificial
  VIM-2 variant
VDSSGEYPTVSEIPVGEVRLYQIADGVWSHIATQSFDGAVYPSNGLIVRDGDELLLIDTAWGAKNTAALLAEIEKQIGLPVTRAVSTHFHDDRVGGVDVLRAAGVATYASPSTRRLAEVEGNEIPTHSLEGLSSSGDAVRFGPVELFYPGAAHSTDNLVVYVPSASVLYGGCAIYELSRTSAGNVADADLAEWPTSIERIQQHYPEAQFVIPGHGLPGGLDLLKHTTNVVKAHTN

SEQ ID NO: 22 - protein, 235 aa, artificial
  VIM-2 variant
VDSSGEYPTVSEIPVGEVRLYQIADGVWSHIATRSFDGAVYPSNGLIVRDGDELLLIDTAWGAKNTAALLAEIEKQIGLPVTRAVSTHFHDDRVGGVDVLRAAGVATYASPSTRRLAEVEGNEIPTHSLEGLSSSGDAVRFGPVELFYPGAAHSTDNLVVYVPSASVLYGGCAIYELSRTSAGNVADADLAEWPTSIERIQQHYPEAQFVIPGHGLPGGLDLLKHTTNVVKAHTN

SEQ ID NO: 23 - protein, 240 aa, artificial
  VIM-2  Q34R Q22H
VDSSGEYPTVSEIPVGEVRLYHIADGVWSHIATRSFDGAVYPSNGLIVRDGDELLLIDTAWGAKNTAALLAEIEKQIGLPVTRAVSTHFHDDRVGGVDVLRAAGVATYASPSTRRLAEVEGNEIPTHSLEGLSSSGDAVRFGPVELFYPGAAHSTDNLVVYVPSASVLYGGCAIYELSRTSAGNVADADLAEWPTSIERIQQHYPEAQFVIPGHGLPGGLDLLKHTTNVVKAHTNRSVVE

SEQ ID NO: 24 - protein, 240 aa, artificial
  VIM-2  Q34R Q22N
VDSSGEYPTVSEIPVGEVRLYNIADGVWSHIATRSFDGAVYPSNGLIVRDGDELLLIDTAWGAKNTAALLAEIEKQIGLPVTRAVSTHFHDDRVGGVDVLRAAGVATYASPSTRRLAEVEGNEIPTHSLEGLSSSGDAVRFGPVELFYPGAAHSTDNLVVYVPSASVLYGGCAIYELSRTSAGNVADADLAEWPTSIERIQQHYPEAQFVIPGHGLPGGLDLLKHTTNVVKAHTNRSVVE

SEQ ID NO: 25 - protein, 240 aa, artificial
  VIM-2  Q34R E130D
VDSSGEYPTVSEIPVGEVRLYQIADGVWSHIATRSFDGAVYPSNGLIVRDGDELLLIDTAWGAKNTAALLAEIEKQIGLPVTRAVSTHFHDDRVGGVDVLRAAGVATYASPSTRRLAEVEGNEIPTHSLDGLSSSGDAVRFGPVELFYPGAAHSTDNLVVYVPSASVLYGGCAIYELSRTSAGNVADADLAEWPTSIERIQQHYPEAQFVIPGHGLPGGLDLLKHTTNVVKAHTNRSVVE

SEQ ID NO: 26 - protein, 240 aa, artificial
  VIM-2  Q34R E130D Q22N
VDSSGEYPTVSEIPVGEVRLYNIADGVWSHIATRSFDGAVYPSNGLIVRDGDELLLIDTAWGAKNTAALLAEIEKQIGLPVTRAVSTHFHDDRVGGVDVLRAAGVATYASPSTRRLAEVEGNEIPTHSLDGLSSSGDAVRFGPVELFYPGAAHSTDNLVVYVPSASVLYGGCAIYELSRTSAGNVADADLAEWPTSIERIQQHYPEAQFVIPGHGLPGGLDLLKHTTNVVKAHTNRSVVE

SEQ ID NO: 27 - protein, 240 aa, artificial
  VIM-2  Q34R E130D Q22H
VDSSGEYPTVSEIPVGEVRLYHIADGVWSHIATRSFDGAVYPSNGLIVRDGDELLLIDTAWGAKNTAALLAEIEKQIGLPVTRAVSTHFHDDRVGGVDVLRAAGVATYASPSTRRLAEVEGNEIPTHSLDGLSSSGDAVRFGPVELFYPGAAHSTDNLVVYVPSASVLYGGCAIYELSRTSAGNVADADLAEWPTSIERIQQHYPEAQFVIPGHGLPGGLDLLKHTTNVVKAHTNRSVVE

SEQ ID NO: 28 - protein, 235 aa, artificial
  VIM-2  Q34R Q22H DCT236
VDSSGEYPTVSEIPVGEVRLYHIADGVWSHIATRSFDGAVYPSNGLIVRDGDELLLIDTAWGAKNTAALLAEIEKQIGLPVTRAVSTHFHDDRVGGVDVLRAAGVATYASPSTRRLAEVEGNEIPTHSLEGLSSSGDAVRFGPVELFYPGAAHSTDNLVVYVPSASVLYGGCAIYELSRTSAGNVADADLAEWPTSIERIQQHYPEAQFVIPGHGLPGGLDLLKHTTNVVKAHTN

SEQ ID NO: 29 - protein, 235 aa, artificial
  VIM-2  Q34R Q22N DCT236
VDSSGEYPTVSEIPVGEVRLYNIADGVWSHIATRSFDGAVYPSNGLIVRDGDELLLIDTAWGAKNTAALLAEIEKQIGLPVTRAVSTHFHDDRVGGVDVLRAAGVATYASPSTRRLAEVEGNEIPTHSLEGLSSSGDAVRFGPVELFYPGAAHSTDNLVVYVPSASVLYGGCAIYELSRTSAGNVADADLAEWPTSIERIQQHYPEAQFVIPGHGLPGGLDLLKHTTNVVKAHTN

SEQ ID NO: 30 - protein, 235 aa, artificial
  VIM-2  Q34R E130D DCT236
VDSSGEYPTVSEIPVGEVRLYQIADGVWSHIATRSFDGAVYPSNGLIVRDGDELLLIDTAWGAKNTAALLAEIEKQIGLPVTRAVSTHFHDDRVGGVDVLRAAGVATYASPSTRRLAEVEGNEIPTHSLDGLSSSGDAVRFGPVELFYPGAAHSTDNLVVYVPSASVLYGGCAIYELSRTSAGNVADADLAEWPTSIERIQQHYPEAQFVIPGHGLPGGLDLLKHTTNVVKAHTN

SEQ ID NO: 31 - protein, 235 aa, artificial
  VIM-2  Q34R E130D Q22N DCT236
VDSSGEYPTVSEIPVGEVRLYNIADGVWSHIATRSFDGAVYPSNGLIVRDGDELLLIDTAWGAKNTAALLAEIEKQIGLPVTRAVSTHFHDDRVGGVDVLRAAGVATYASPSTRRLAEVEGNEIPTHSLDGLSSSGDAVRFGPVELFYPGAAHSTDNLVVYVPSASVLYGGCAIYELSRTSAGNVADADLAEWPTSIERIQQHYPEAQFVIPGHGLPGGLDLLKHTTNVVKAHTN

SEQ ID NO: 32 - protein, 235 aa, artificial
  VIM-2  Q34R E130D Q22H DCT236
VDSSGEYPTVSEIPVGEVRLYHIADGVWSHIATRSFDGAVYPSNGLIVRDGDELLLIDTAWGAKNTAALLAEIEKQIGLPVTRAVSTHFHDDRVGGVDVLRAAGVATYASPSTRRLAEVEGNEIPTHSLDGLSSSGDAVRFGPVELFYPGAAHSTDNLVVYVPSASVLYGGCAIYELSRTSAGNVADADLAEWPTSIERIQQHYPEAQFVIPGHGLPGGLDLLKHTTNVVKAHTN

SEQ ID NO: 33 - protein, 240 aa, artificial
  VIM-2  V1M Q34R Q22H
MDSSGEYPTVSEIPVGEVRLYHIADGVWSHIATRSFDGAVYPSNGLIVRDGDELLLIDTAWGAKNTAALLAEIEKQIGLPVTRAVSTHFHDDRVGGVDVLRAAGVATYASPSTRRLAEVEGNEIPTHSLEGLSSSGDAVRFGPVELFYPGAAHSTDNLVVYVPSASVLYGGCAIYELSRTSAGNVADADLAEWPTSIERIQQHYPEAQFVIPGHGLPGGLDLLKHTTNVVKAHTNRSVVE

SEQ ID NO: 34 - protein, 240 aa, artificial
  VIM-2  V1M Q34R Q22N
MDSSGEYPTVSEIPVGEVRLYNIADGVWSHIATRSFDGAVYPSNGLIVRDGDELLLIDTAWGAKNTAALLAEIEKQIGLPVTRAVSTHFHDDRVGGVDVLRAAGVATYASPSTRRLAEVEGNEIPTHSLEGLSSSGDAVRFGPVELFYPGAAHSTDNLVVYVPSASVLYGGCAIYELSRTSAGNVADADLAEWPTSIERIQQHYPEAQFVIPGHGLPGGLDLLKHTTNVVKAHTNRSVVE

SEQ ID NO: 35 - protein, 240 aa, artificial
  VIM-2  V1M Q34R E130D
MDSSGEYPTVSEIPVGEVRLYQIADGVWSHIATRSFDGAVYPSNGLIVRDGDELLLIDTAWGAKNTAALLAEIEKQIGLPVTRAVSTHFHDDRVGGVDVLRAAGVATYASPSTRRLAEVEGNEIPTHSLDGLSSSGDAVRFGPVELFYPGAAHSTDNLVVYVPSASVLYGGCAIYELSRTSAGNVADADLAEWPTSIERIQQHYPEAQFVIPGHGLPGGLDLLKHTTNVVKAHTNRSVVE

SEQ ID NO: 36 - protein, 240 aa, artificial
  VIM-2  V1M Q34R E130D Q22N
MDSSGEYPTVSEIPVGEVRLYNIADGVWSHIATRSFDGAVYPSNGLIVRDGDELLLIDTAWGAKNTAALLAEIEKQIGLPVTRAVSTHFHDDRVGGVDVLRAAGVATYASPSTRRLAEVEGNEIPTHSLDGLSSSGDAVRFGPVELFYPGAAHSTDNLVVYVPSASVLYGGCAIYELSRTSAGNVADADLAEWPTSIERIQQHYPEAQFVIPGHGLPGGLDLLKHTTNVVKAHTNRSVVE

SEQ ID NO: 37 - protein, 240 aa, artificial
  VIM-2  V1M Q34R E130D Q22H
MDSSGEYPTVSEIPVGEVRLYHIADGVWSHIATRSFDGAVYPSNGLIVRDGDELLLIDTAWGAKNTAALLAEIEKQIGLPVTRAVSTHFHDDRVGGVDVLRAAGVATYASPSTRRLAEVEGNEIPTHSLDGLSSSGDAVRFGPVELFYPGAAHSTDNLVVYVPSASVLYGGCAIYELSRTSAGNVADADLAEWPTSIERIQQHYPEAQFVIPGHGLPGGLDLLKHTTNVVKAHTNRSVVE

SEQ ID NO: 38 - protein, 235 aa, artificial
  VIM-2  V1M Q34R Q22H DCT236
MDSSGEYPTVSEIPVGEVRLYHIADGVWSHIATRSFDGAVYPSNGLIVRDGDELLLIDTAWGAKNTAALLAEIEKQIGLPVTRAVSTHFHDDRVGGVDVLRAAGVATYASPSTRRLAEVEGNEIPTHSLEGLSSSGDAVRFGPVELFYPGAAHSTDNLVVYVPSASVLYGGCAIYELSRTSAGNVADADLAEWPTSIERIQQHYPEAQFVIPGHGLPGGLDLLKHTTNVVKAHTN

SEQ ID NO: 39 - protein, 235 aa, artificial
  VIM-2  V1M Q34R Q22N DCT236
MDSSGEYPTVSEIPVGEVRLYNIADGVWSHIATRSFDGAVYPSNGLIVRDGDELLLIDTAWGAKNTAALLAEIEKQIGLPVTRAVSTHFHDDRVGGVDVLRAAGVATYASPSTRRLAEVEGNEIPTHSLEGLSSSGDAVRFGPVELFYPGAAHSTDNLVVYVPSASVLYGGCAIYELSRTSAGNVADADLAEWPTSIERIQQHYPEAQFVIPGHGLPGGLDLLKHTTNVVKAHTN

SEQ ID NO: 40 - protein, 235 aa, artificial
  VIM-2  V1M Q34R E130D DCT236
MDSSGEYPTVSEIPVGEVRLYQIADGVWSHIATRSFDGAVYPSNGLIVRDGDELLLIDTAWGAKNTAALLAEIEKQIGLPVTRAVSTHFHDDRVGGVDVLRAAGVATYASPSTRRLAEVEGNEIPTHSLDGLSSSGDAVRFGPVELFYPGAAHSTDNLVVYVPSASVLYGGCAIYELSRTSAGNVADADLAEWPTSIERIQQHYPEAQFVIPGHGLPGGLDLLKHTTNVVKAHTN

SEQ ID NO: 41 - protein, 235 aa, artificial
  VIM-2  V1M Q34R E130D Q22N DCT236
MDSSGEYPTVSEIPVGEVRLYNIADGVWSHIATRSFDGAVYPSNGLIVRDGDELLLIDTAWGAKNTAALLAEIEKQIGLPVTRAVSTHFHDDRVGGVDVLRAAGVATYASPSTRRLAEVEGNEIPTHSLDGLSSSGDAVRFGPVELFYPGAAHSTDNLVVYVPSASVLYGGCAIYELSRTSAGNVADADLAEWPTSIERIQQHYPEAQFVIPGHGLPGGLDLLKHTTNVVKAHTN

SEQ ID NO: 42 - protein, 235 aa, artificial
  VIM-2  V1M Q34R E130D Q22H DCT236
MDSSGEYPTVSEIPVGEVRLYHIADGVWSHIATRSFDGAVYPSNGLIVRDGDELLLIDTAWGAKNTAALLAEIEKQIGLPVTRAVSTHFHDDRVGGVDVLRAAGVATYASPSTRRLAEVEGNEIPTHSLDGLSSSGDAVRFGPVELFYPGAAHSTDNLVVYVPSASVLYGGCAIYELSRTSAGNVADADLAEWPTSIERIQQHYPEAQFVIPGHGLPGGLDLLKHTTNVVKAHTN

SEQ ID NO: 43 - protein, 240 aa, artificial
  VIM-2 V10A
VDSSGEYPTASEIPVGEVRLYQIADGVWSHIATQSFDGAVYPSNGLIVRDGDELLLIDTAWGAKNTAALLAEIEKQIGLPVTRAVSTHFHDDRVGGVDVLRAAGVATYASPSTRRLAEVEGNEIPTHSLEGLSSSGDAVRFGPVELFYPGAAHSTDNLVVYVPSASVLYGGCAIYELSRTSAGNVADADLAEWPTSIERIQQHYPEAQFVIPGHGLPGGLDLLKHTTNVVKAHTNRSVVE

SEQ ID NO: 44 - protein, 240 aa, artificial
  VIM-2 V10A Q34R Q22H
VDSSGEYPTASEIPVGEVRLYHIADGVWSHIATRSFDGAVYPSNGLIVRDGDELLLIDTAWGAKNTAALLAEIEKQIGLPVTRAVSTHFHDDRVGGVDVLRAAGVATYASPSTRRLAEVEGNEIPTHSLEGLSSSGDAVRFGPVELFYPGAAHSTDNLVVYVPSASVLYGGCAIYELSRTSAGNVADADLAEWPTSIERIQQHYPEAQFVIPGHGLPGGLDLLKHTTNVVKAHTNRSVVE

SEQ ID NO: 45 - protein, 240 aa, artificial
  VIM-2 V10A Q34R Q22N
VDSSGEYPTASEIPVGEVRLYNIADGVWSHIATRSFDGAVYPSNGLIVRDGDELLLIDTAWGAKNTAALLAEIEKQIGLPVTRAVSTHFHDDRVGGVDVLRAAGVATYASPSTRRLAEVEGNEIPTHSLEGLSSSGDAVRFGPVELFYPGAAHSTDNLVVYVPSASVLYGGCAIYELSRTSAGNVADADLAEWPTSIERIQQHYPEAQFVIPGHGLPGGLDLLKHTTNVVKAHTNRSVVE

SEQ ID NO: 46 - protein, 240 aa, artificial
  VIM-2 V10A Q34R E130D
VDSSGEYPTASEIPVGEVRLYQIADGVWSHIATRSFDGAVYPSNGLIVRDGDELLLIDTAWGAKNTAALLAEIEKQIGLPVTRAVSTHFHDDRVGGVDVLRAAGVATYASPSTRRLAEVEGNEIPTHSLDGLSSSGDAVRFGPVELFYPGAAHSTDNLVVYVPSASVLYGGCAIYELSRTSAGNVADADLAEWPTSIERIQQHYPEAQFVIPGHGLPGGLDLLKHTTNVVKAHTNRSVVE

SEQ ID NO: 47 - protein, 240 aa, artificial
  VIM-2 V10A Q34R E130D Q22N
VDSSGEYPTASEIPVGEVRLYNIADGVWSHIATRSFDGAVYPSNGLIVRDGDELLLIDTAWGAKNTAALLAEIEKQIGLPVTRAVSTHFHDDRVGGVDVLRAAGVATYASPSTRRLAEVEGNEIPTHSLDGLSSSGDAVRFGPVELFYPGAAHSTDNLVVYVPSASVLYGGCAIYELSRTSAGNVADADLAEWPTSIERIQQHYPEAQFVIPGHGLPGGLDLLKHTTNVVKAHTNRSVVE

SEQ ID NO: 48 - protein, 240 aa, artificial
  VIM-2 V10A Q34R E130D Q22H
VDSSGEYPTASEIPVGEVRLYHIADGVWSHIATRSFDGAVYPSNGLIVRDGDELLLIDTAWGAKNTAALLAEIEKQIGLPVTRAVSTHFHDDRVGGVDVLRAAGVATYASPSTRRLAEVEGNEIPTHSLDGLSSSGDAVRFGPVELFYPGAAHSTDNLVVYVPSASVLYGGCAIYELSRTSAGNVADADLAEWPTSIERIQQHYPEAQFVIPGHGLPGGLDLLKHTTNVVKAHTNRSVVE

SEQ ID NO: 49 - protein, 235 aa, artificial
  VIM-2 V10A Q34R Q22H DCT236
VDSSGEYPTASEIPVGEVRLYHIADGVWSHIATRSFDGAVYPSNGLIVRDGDELLLIDTAWGAKNTAALLAEIEKQIGLPVTRAVSTHFHDDRVGGVDVLRAAGVATYASPSTRRLAEVEGNEIPTHSLEGLSSSGDAVRFGPVELFYPGAAHSTDNLVVYVPSASVLYGGCAIYELSRTSAGNVADADLAEWPTSIERIQQHYPEAQFVIPGHGLPGGLDLLKHTTNVVKAHTN

SEQ ID NO: 50 - protein, 235 aa, artificial
  VIM-2 V10A Q34R Q22N DCT236 (
VDSSGEYPTASEIPVGEVRLYNIADGVWSHIATRSFDGAVYPSNGLIVRDGDELLLIDTAWGAKNTAALLAEIEKQIGLPVTRAVSTHFHDDRVGGVDVLRAAGVATYASPSTRRLAEVEGNEIPTHSLEGLSSSGDAVRFGPVELFYPGAAHSTDNLVVYVPSASVLYGGCAIYELSRTSAGNVADADLAEWPTSIERIQQHYPEAQFVIPGHGLPGGLDLLKHTTNVVKAHTN

SEQ ID NO: 51 - protein, 235 aa, artificial
  VIM-2 V10A Q34R E130D DCT236
VDSSGEYPTASEIPVGEVRLYQIADGVWSHIATRSFDGAVYPSNGLIVRDGDELLLIDTAWGAKNTAALLAEIEKQIGLPVTRAVSTHFHDDRVGGVDVLRAAGVATYASPSTRRLAEVEGNEIPTHSLDGLSSSGDAVRFGPVELFYPGAAHSTDNLVVYVPSASVLYGGCAIYELSRTSAGNVADADLAEWPTSIERIQQHYPEAQFVIPGHGLPGGLDLLKHTTNVVKAHTN

SEQ ID NO: 52 - protein, 235 aa, artificial
  VIM-2 V10A Q34R E130D Q22N DCT236
VDSSGEYPTASEIPVGEVRLYNIADGVWSHIATRSFDGAVYPSNGLIVRDGDELLLIDTAWGAKNTAALLAEIEKQIGLPVTRAVSTHFHDDRVGGVDVLRAAGVATYASPSTRRLAEVEGNEIPTHSLDGLSSSGDAVRFGPVELFYPGAAHSTDNLVVYVPSASVLYGGCAIYELSRTSAGNVADADLAEWPTSIERIQQHYPEAQFVIPGHGLPGGLDLLKHTTNVVKAHTN

SEQ ID NO: 53 - protein, 235 aa, artificial
  VIM-2 V10A Q34R E130D Q22H DCT236
VDSSGEYPTASEIPVGEVRLYHIADGVWSHIATRSFDGAVYPSNGLIVRDGDELLLIDTAWGAKNTAALLAEIEKQIGLPVTRAVSTHFHDDRVGGVDVLRAAGVATYASPSTRRLAEVEGNEIPTHSLDGLSSSGDAVRFGPVELFYPGAAHSTDNLVVYVPSASVLYGGCAIYELSRTSAGNVADADLAEWPTSIERIQQHYPEAQFVIPGHGLPGGLDLLKHTTNVVKAHTN

SEQ ID NO: 54 - protein, 240 aa, artificial
  VIM-2 V10A Q34R E130D Q22H DCT236
MDSSGEYPTASEIPVGEVRLYHIADGVWSHIATRSFDGAVYPSNGLIVRDGDELLLIDTAWGAKNTAALLAEIEKQIGLPVTRAVSTHFHDDRVGGVDVLRAAGVATYASPSTRRLAEVEGNEIPTHSLEGLSSSGDAVRFGPVELFYPGAAHSTDNLVVYVPSASVLYGGCAIYELSRTSAGNVADADLAEWPTSIERIQQHYPEAQFVIPGHGLPGGLDLLKHTTNVVKAHTNRSVVE

SEQ ID NO: 55 - protein, 240 aa, artificial
  VIM-2 V10A V1M Q34R Q22N
MDSSGEYPTASEIPVGEVRLYNIADGVWSHIATRSFDGAVYPSNGLIVRDGDELLLIDTAWGAKNTAALLAEIEKQIGLPVTRAVSTHFHDDRVGGVDVLRAAGVATYASPSTRRLAEVEGNEIPTHSLEGLSSSGDAVRFGPVELFYPGAAHSTDNLVVYVPSASVLYGGCAIYELSRTSAGNVADADLAEWPTSIERIQQHYPEAQFVIPGHGLPGGLDLLKHTTNVVKAHTNRSVVE

SEQ ID NO: 56 - protein, 240 aa, artificial
  VIM-2 V10A V1M Q34R E130D
MDSSGEYPTASEIPVGEVRLYQIADGVWSHIATRSFDGAVYPSNGLIVRDGDELLLIDTAWGAKNTAALLAEIEKQIGLPVTRAVSTHFHDDRVGGVDVLRAAGVATYASPSTRRLAEVEGNEIPTHSLDGLSSSGDAVRFGPVELFYPGAAHSTDNLVVYVPSASVLYGGCAIYELSRTSAGNVADADLAEWPTSIERIQQHYPEAQFVIPGHGLPGGLDLLKHTTNVVKAHTNRSVVE

SEQ ID NO: 57 - protein, 240 aa, artificial
  VIM-2 V10A V1M Q34R E130D Q22N
MDSSGEYPTASEIPVGEVRLYNIADGVWSHIATRSFDGAVYPSNGLIVRDGDELLLIDTAWGAKNTAALLAEIEKQIGLPVTRAVSTHFHDDRVGGVDVLRAAGVATYASPSTRRLAEVEGNEIPTHSLDGLSSSGDAVRFGPVELFYPGAAHSTDNLVVYVPSASVLYGGCAIYELSRTSAGNVADADLAEWPTSIERIQQHYPEAQFVIPGHGLPGGLDLLKHTTNVVKAHTNRSVVE

SEQ ID NO: 58 - protein, 240 aa, artificial
  VIM-2 V10A V1M Q34R E130D Q22H
MDSSGEYPTASEIPVGEVRLYHIADGVWSHIATRSFDGAVYPSNGLIVRDGDELLLIDTAWGAKNTAALLAEIEKQIGLPVTRAVSTHFHDDRVGGVDVLRAAGVATYASPSTRRLAEVEGNEIPTHSLDGLSSSGDAVRFGPVELFYPGAAHSTDNLVVYVPSASVLYGGCAIYELSRTSAGNVADADLAEWPTSIERIQQHYPEAQFVIPGHGLPGGLDLLKHTTNVVKAHTNRSVVE

SEQ ID NO: 59 - protein, 235 aa, artificial
  VIM-2 V10A V1M Q34R Q22H DCT236
MDSSGEYPTASEIPVGEVRLYHIADGVWSHIATRSFDGAVYPSNGLIVRDGDELLLIDTAWGAKNTAALLAEIEKQIGLPVTRAVSTHFHDDRVGGVDVLRAAGVATYASPSTRRLAEVEGNEIPTHSLEGLSSSGDAVRFGPVELFYPGAAHSTDNLVVYVPSASVLYGGCAIYELSRTSAGNVADADLAEWPTSIERIQQHYPEAQFVIPGHGLPGGLDLLKHTTNVVKAHTN

SEQ ID NO: 60 - protein, 235 aa, artificial
  VIM-2 V10A V1M Q34R Q22N DCT236
MDSSGEYPTASEIPVGEVRLYNIADGVWSHIATRSFDGAVYPSNGLIVRDGDELLLIDTAWGAKNTAALLAEIEKQIGLPVTRAVSTHFHDDRVGGVDVLRAAGVATYASPSTRRLAEVEGNEIPTHSLEGLSSSGDAVRFGPVELFYPGAAHSTDNLVVYVPSASVLYGGCAIYELSRTSAGNVADADLAEWPTSIERIQQHYPEAQFVIPGHGLPGGLDLLKHTTNVVKAHTN

SEQ ID NO: 61 - protein, 235 aa, artificial
  VIM-2 V10A V1M Q34R E130D DCT236
MDSSGEYPTASEIPVGEVRLYQIADGVWSHIATRSFDGAVYPSNGLIVRDGDELLLIDTAWGAKNTAALLAEIEKQIGLPVTRAVSTHFHDDRVGGVDVLRAAGVATYASPSTRRLAEVEGNEIPTHSLDGLSSSGDAVRFGPVELFYPGAAHSTDNLVVYVPSASVLYGGCAIYELSRTSAGNVADADLAEWPTSIERIQQHYPEAQFVIPGHGLPGGLDLLKHTTNVVKAHTN

SEQ ID NO: 62 - protein, 235 aa, artificial
  VIM-2 V10A V1M Q34R E130D Q22N DCT236
MDSSGEYPTASEIPVGEVRLYNIADGVWSHIATRSFDGAVYPSNGLIVRDGDELLLIDTAWGAKNTAALLAEIEKQIGLPVTRAVSTHFHDDRVGGVDVLRAAGVATYASPSTRRLAEVEGNEIPTHSLDGLSSSGDAVRFGPVELFYPGAAHSTDNLVVYVPSASVLYGGCAIYELSRTSAGNVADADLAEWPTSIERIQQHYPEAQFVIPGHGLPGGLDLLKHTTNVVKAHTN

SEQ ID NO: 63 - protein, 263 aa, artificial
  P1A
EMKDDFAKLEEQFDAKLGIFALDTGTNRTVAYRPDERFAFASTIKALTVGVLLQQKSIEDLNQRITYTRDDLVNYNPITEKHVDTGMTLKELADASLRYSDNAAQNLILKQIGGPESLKKELRKIGDEVTNPERFEPELNEVNPGETQDTSTARALVTSLRAFALEDKLPSEKRELLIDWMKRNTTGDALIRAGVPDGWEVADKTGAASYGTRNDIAIIWPPKGDPVVLAVLSSRDKKDAKYDDKLIAEATKVVMKALNMNGK

SEQ ID NO: 64 - protein, 215 aa, artificial
  P2A
ETGTISISQLNKNVWVHTELGYFNGEAVPSNGLVLNTSKGLVLVDSSWDNKLTKELIEMVEKKFQKRVTDVIITHAHADRIGGITALKERGIKAHSTALTAELAKNSGYEEPLGDLQTITSLKFGNTKVETFYPGKGHTEDNIVVWLPQYQILAGGCLVKSAEAKDLGNVADAYVNEWSTSIENVLKRYGNINSWPGHGEVGDKGLLLHTLDLLK

SEQ ID NO: 65 - protein, 299 aa, artificial
  KPC-1/2
MIQKRKRTVSFRLVLMCTLLFVSLPITKTSAQASKTEMKDDFAKLEEQFDAKLGIFALDTGTNRTVAYRPDERFAFASTIKALTVGVLLQQKSIEDLNQRITYTRDDLVNYNPITEKHVDTGMTLKELADASLRYSDNAAQNLILKQIGGPESLKKELRKIGDEVTNPERFEPELNEVNPGETQDTSTARALVTSLRAFALEDKLPSEKRELLIDWMKRNTTGDALIRAGVPDGWEVGDKTGSGDYGTRNDIAIIWPPKGDPVVLAVLSSRDKKDAKYDNKLIAEATKVVMKALNMNGK

SEQ ID NO: 66 - protein, 293 aa, artificial
  KPC-3
MSLYRRLVLLSCLSWPLAGFSATALTNLVAEPFAKLEQDFGGSIGVYAMDTGSGATVSYRAEERFPLCSSFKGFLAAAVLARSQQQAGLLDTPIRYGKNALVPWSPISEKYLTTGMTVAELSAAAVQYSDNAAANLLLKELGGPAGLTAFMRSIGDTTFRLDRWELELNSAIPGDARDTSSPRAVTESLQKLTLGSALAAPQRQQFVDWLKGNTTGNHRIRAAVPADWAVGDKTGTCGVYGTANDYAVVWPTGRAPIVLAVYTRAPNKDDKYSEAVIAAAARLALEGLGVNGQ

SEQ ID NO: 67 - protein, 293 aa, artificial; identical to SEQ ID NO: 66
  KPC-4

SEQ ID NO: 68 - protein, 293 aa, artificial
  KPC-5
MSLYRRLVLLSCLSWPLAGFSATALTNLVAEPFAKLEQDFGGSIGVYAMDTGSGATVSYRAEERFPLCSSFKGFLAAAVLARSQQQAGLLDTPIRYGKNALVRWSPISEKYLTTGMTVAELSAAAVQYSDNAAANLLLKELGGPAGLTAFMRSIGDTTFRLDRWELELNSAIPGDARDTSSPRAVTESLQKLTLGSALAAPQRQQFVDWLKGNTTGNHRIRAAVPADWAVGDKTGTCGVYGTANDYAVVWPTGRAPIVLAVYTRAPNKDDKHSEAVIAAAARLALEGLGVNGQ

SEQ ID NO: 69 - protein, 292 aa, artificial
  KPC-6
MSLYRRLVLLSCLSWPLAGFSATALTNLVAEPFAKLEQDFGGSIGVYAMDTGSGATVSYRAEERFPLCSSFKGFLAAAVLARSQQQAGLLDTPIRYGKNALVPWSPISEKYLTTGMTVAELSAAAVQYSDNAAANLLLKELGGPAGLTAFMRSIGDTTFRLDRWELELNSAIPGDARDTSSPRAVTESLQKLTLGSALAAPQRQQFVDWLKGNTTGNHRIRAAVPADWAVGDKTGTCGGYGTANDYAWWPTGRAPIVLAVYTRAPNKDDKHSEAVIAAAARLALEGLGVNGQ

SEQ ID NO: 70 - protein, 293 aa, artificial
  KPC-7
MSLYRRLVLLSCLSWPLAGFSATALTNLVAEPFAKLEQDFGGSIGVYAIDTGSGATVSYRAEERFPLCSSFKGFLAAAVLARSQQQAGLLDTPIRYGKNALVPWSPISEKYLTTGMTVAELSAAAVQYSDNAAANLLLKELGGPAGLTAFMRSIGDTTFRLDRWELELNSAIPGDARDTSSPRAVTESLQKLTLGSALAAPQRQQFVDWLKGNTTGNHRLRAAVPADWAVGDKTGTCGVYGTANDYAVVWPTGRAPIVLAVYTRAPNKDDKYSEAVIAAAARLALEGLGVNGQ

SEQ ID NO: 71 - protein, 292 aa, artificial
  KPC-8
MSLYRRLVLLSCLSWPLAGFSATALTNLVAEPFAKLEQDFGGSIGVYAMDTGSGATVSYRAEERFPLCSSFKGFLAAAVLARSQQQAGLLDTPIRYGKNALVPWSPISEKYLTTGMTVAELSAAAVQYSDNAAANLLLKELGGPAGLTAFMRSIGDTTFRLDRWELELNSAIPGDARDTSSPRAVTESLQKLTLGSALAAPQRQQFVDWLKGNTTGNHRIRAAVPADWAVGDKTGTCGGYGTANDYAWWPTGRAPIVLAVYTRAPNKDDKYSEAVIAAAARLALEGLGVNGQ

SEQ ID NO: 72 - protein, 293 aa, artificial
  KPC-9
MSKYRRLVLLSCLSWPLAGFSATALTNLVAEPFAKLEQDFGGSIGVYAMDTGSGATVSYRAEERFPLCSSFKGFLAAAVLARSQQQAGLLDTPIRYGKNALVPWSPISEKYLTTGMTVAELSAAAVQYSDNAAANLLLKELGGPAGLTAFMRSIGDTTFRLDRWELELNSAIPGDARDTSSPRAVTESLQKLTLGSALAAPQRQQFVDWLKGNTTGNHRIRAAVPADWAVGDKTGTCGAYGTANDYAVVWPTGRAPIVLAVYTRAPNKDDKYSEAVIAAAARLALEGLGVNGQ

SEQ ID NO: 73 - protein, 293 aa, artificial
  KPC-10
MSLYRRLVLLSCLSWPLAGFSATALTNLVAEPFAKLEQDFGGSIGVYAMDTGSGATVSYRAEERFPLCSSFKGFLAAAVLARSQQQAGLLDTPIRYGKNALVRWSPISEKYLTTGMTVAELSAAAVQYSDNAAANLLLKELGGPAGLTAFMRSIGDTTFRLDRWELELNSAIPGDARDTSSPRAVTESLQKLTLGSALAAPQRQQFVDWLKGNTTGNHRIRAAVPADWAVGDKTGTCGVYGTANDYAVVWPTGRAPIVLAVYTRAPNKDDKYSEAVIAAAARLALEGLGVNGQ

SEQ ID NO: 74 - protein, 293 aa, artificial
  KPC-11
MSLYRRLVLLSCLSWPLAGFSATALTNLVAEPFAKLEQDFGGSIGVYAMDTGSGATVSYRAEERFPLCSSFKGFLAAAVLARSQQQAGLLDTPIRYGKNALVLWSPISEKYLTTGMTVAELSAAAVQYSDNAAANLLLKELGGPAGLTAFMRSIGDTTFRLDRWELELNSAIPGDARDTSSPRAVTESLQKLTLGSALAAPQRQQFVDWLKGNTTGNHRIRAAVPADWAVGDKTGTCGVYGTANDYAVVWPTGRAPIVLAVYTRAPNKDDKHSEAVIAAAARLALEGLGVNGQ

SEQ ID NO: 75 - protein, 293 aa, artificial
  KPC-12
MSLYRRLVLLSCLSWPLAGFSATALTNLVAEPFAKLEQDFGGSIGVYAMDTGSGATVSYRAEERFPLCSSFKGFLAAAVLARSQQQAGLLDTPIRYGKNALVPWSPISEKYLTTGMTVAELSAAAVQYSDNAAANLLLKELGGPAGLTAFMRSIGDTTFRLDRWELEMNSAIPGDARDTSSPRAVTESLQKLTLGSALAAPQRQQFVDWLKGNTTGNHRIRAAVPADWAVGDKTGTCGVYGTANDYAVVWPTGRAPIVLAVYTRAPNKDDKHSEAVIAAAARLALEGLGVNGQ

SEQ ID NO: 76 - protein, 293 aa, artificial
  KPC-13
MSLYRRLVLLSCLSWPLAGFSATALTNLVAEPFAKLEQDFGGSIGVYAMDTGSGATVSYRAEERFPLCSSFKGFLAAAVLARSQQQAGLLGTPIRYGKNALVPWSPISEKYLTTGMTVAELSAAAVQYSDNAAANLLLKELGGPAGLTAFMRSIGDTTFRLDRWELELNSAIPGDARDTSSPRAVTESLQKLTLGSALAAPQRQQFVDWLKGNTTGNHRIRAAVPADWAVGDKTGTCGVYGTANDYAVVWPTGRAPIVLAVYTRAPNKDDKYSEAVIAAAARLALEGLGVNGQ

SEQ ID NO: 77 - protein, 291 aa, artificial
  KPC-14
MSLYRRLVLLSCLSWPLAGFSATALTNLVAEPFAKLEQDFGGSIGVYAMDTGSGATVSYRAEERFPLCSSFKGFLAAAVLARSQQQAGLLDTPIRYGKNALVPWSPISEKYLTTGMTVAELSAAAVQYSDNAAANLLLKELGGPAGLTAFMRSIGDTTFRLDRWELELNSAIPGDARDTSSPRAVTESLQKLTLGSALAAPQRQQFVDWLKGNTTGNHRIRAAVPADWAVGDKTGTCGVYANDYAVVWPTGRAPIVLAVYTRAPNKDDKHSEAVIAAAARLALEGLGVNGQ

SEQ ID NO: 78 - protein, 292 aa, artificial
  KPC-15
MSLYRRLVLLSCLSWPLAGFSATALTNLVAEPFAKLEQDFGGSIGVYAMDTGSGATVSYRAEERFPLCSSFKGFLAAAVLARSQQQAGLLDTPIRYGKNALVRWSPISEKYLTTGMTVLELSAAAVQYSDNAAANLLLKELGGPAKLTAFMRSIGDTTFRLDRWELELNSAIPGDARDTSSPRAVTESLQKLTLGSALAAPQRQQFVDWLKGNTTGNHRIRAAVPADWAVGDKTGTCGGYGTANDYAWWPTGRAPIVLAVYTRAPNKDDKYSEAVIAAAARLALEGLGVNGQ

SEQ ID NO: 79 - protein, 293 aa, artificial
  KPC-17
MSLYRRLVLLSCLSWPLAGFSATALTNLVAEPFAKLEQDFGGSIGVYAMDTGSGATVSYRAEERFPLCSSFKGFLAAAVLARSQQQAGLLDTPIRYGKNALVPWSPISEKYLTTGMTVAELSAAAVQYSDNAAANLLLKELGGPAGLTAFMRSIGDTTFRLDRWELELNSAIPGDARDTSSPRAVTESLQKLTLGSALAAPQRQQLVDWLKGNTTGNHRIRAAVPADWAVGDKTGTCGVYGTANDYAVVWPTGRAPIVLAVYTRAPNKDDKHSEAVIAAAARLALEGLGVNGQ

SEQ ID NO: 80 - protein, 269 aa, artificial
  NDM-1
MELPNIMHPVAKLSTALAAALMLSGCMPGEIRPTIGQQMETGDQRFGDLVFRQLAPNVWQHTSYLDMPGFGAVASNGLIVRDGGRVLVVDTAWTDDQTAQILNWIKQEINLPVALAWTHAHQDKMGGMDALHAAGIATYANALSNQLAPQEGMVAAQHSLTFAANGVWEPATAPNFGPLKVFYPGPGHTSDNITVGIDGTDIAFGGCLIKDSKAKSLGNLGDADTEHYAASARAFGAAFPKASMIVMSHSAPDSRAAITHTARMADKLR

SEQ ID NO: 81 - protein, 269 aa, artificial
  NDM-2
MELPNIMHPVAKLSTALAAALMLSGCMAGEIRPTIGQQMETGDQRFGDLVFRQLAPNVWQHTSYLDMPGFGAVASNGLIVRDGGRVLVVDTAWTDDQTAQILNWIKQEINLPVALAWTHAHQDKMGGMDALHAAGIATYANALSNQLAPQEGMVAAQHSLTFAANGVWEPATAPNFGPLKVFYPGPGHTSDNITVGIDGTDIAFGGCLIKDSKAKSLGNLGDADTEHYAASARAFGAAFPKASMIVMSHSAPDSRAAITHTARMADKLR

SEQ ID NO: 82 - protein, 269 aa, artificial
  NDM-3
MELPNIMHPVAKLSTALAAALMLSGCMPGEIRPTIGQQMETGDQRFGDLVFRQLAPNVWQHTSYLDMPGFGAVASNGLIVRDGGRVLVVDTAWTNDQTAQILNWIKQEINLPVALAWTHAHQDKMGGMDALHAAGIATYANALSNQLAPQEGMVAAQHSLTFAANGVWEPATAPNFGPLKVFYPGPGHTSDNITVGIDGTDIAFGGCLIKDSKAKSLGNLGDADTEHYAASARAFGAAFPKASMIVMSHSAPDSRAAITHTARMADKLR

SEQ ID NO: 83 - protein, 268 aa, artificial
  NDM-4
MELPNIMHPVAKLSTALAAALMLSGCMPGEIRPTIGQQMETGDQRFGDLVFRQLAPNVWQHTSYLDMPGFGAVASNGLIVRDGGRVLVVDTAWTDDQTAQILNWIKQEINLPVALAWTHAHQDKMGGMDALHAAGIATYANALSNQLAPQEGLVAAQHSLTFAANGWEPATAPNFGPLKVFYPGPGHTSDNITVGIDGTDIAFGGCLIKDSKAKSLGNLGDADTEHYAASARAFGAAFPKASMIVMSHSAPDSRAAITHTARMADKLR

SEQ ID NO: 84 - protein, 270 aa, artificial
  NDM-5
MELPNIMHPVAKLSTALAAALMLSGCMPGEIRPTIGQQMETGDQRFGDLVFRQLAPNVWQHTSYLDMPGFGAVASNGLIVRDGGRVLLVDTAWTDDQTAQILNWIKQEINLPVALAVVTHAHQDKMGGMDALHAAGIATYANALSNQLAPQEGLVAAQHSLTFAANGVWEPATAPNFGPLKVFYPGPGHTSDNITVGIDGTDIAFGGCLIKDSKAKSLGNLGDADTEHYAASARAFGAAFPKASMIVMSHSAPDSRAAITHTARMADKLR

SEQ ID NO: 85 - protein, 269 aa, artificial
  NDM-6
MELPNIMHPVAKLSTALAAALMLSGCMPGEIRPTIGQQMETGDQRFGDLVFRQLAPNVWQHTSYLDMPGFGAVASNGLIVRDGGRVLVVDTAWTDDQTAQILNWIKQEINLPVALAWTHAHQDKMGGMDALHAAGIATYANALSNQLAPQEGMVAAQHSLTFAANGVWEPATAPNFGPLKVFYPGPGHTSDNITVGIDGTDIAFGGCLIKDSKAKSLGNLGDADTEHYAASVRAFGAAFPKASMIVMSHSAPDSRAAITHTARMADKLR

SEQ ID NO: 86 - protein, 268 aa, artificial
  NDM-7 (
MELPNIMHPVAKLSTALAAALMLSGCMPGEIRPTIGQQMETGDQRFGDLVFRQLAPNVWQHTSYLDMPGFGAVASNGLIVRDGGRVLVVDTAWTDDQTAQILNWIKQEINLPVALAWTHAHQDKMGGMNALHAAGIATYANALSNQLAPQEGLVAAQHSLTFAANGWEPATAPNFGPLKVFYPGPGHTSDNITVGIDGTDIAFGGCLIKDSKAKSLGNLGDADTEHYAASARAFGAAFPKASMIVMSHSAPDSRAAITHTARMADKLR

SEQ ID NO: 87 - protein, 269 aa, artificial
  NDM-8
MELPNIMHPVAKLSTALAAALMLSGCMPGEIRPTIGQQMETGDQRFGDLVFRQLAPNVWQHTSYLDMPGFGAVASNGLIVRDGGRVLVVDTAWTDDQTAQILNWIKQEINLPVALAWTHAHQDKMGGMGALHAAGIATYANALSNQLAPQEGLVAAQHSLTFAANGVWEPATAPNFGPLKVFYPGPGHTSDNITVGIDGTDIAFGGCLIKDSKAKSLGNLGDADTEHYAASARAFGAAFPKASMIVMSHSAPDSRAAITHTARMADKLR

SEQ ID NO: 88 - protein, 268 aa, artificial
  NDM-9
MELPNIMHPVAKLSTALAAALMLSGCMPGEIRPTIGQQMETGDQRFGDLVFRQLAPNVWQHTSYLDMPGFGAVASNGLIVRDGGRVLVVDTAWTDDQTAQILNWIKQEINLPVALAWTHAHQDKMGGMDALHAAGIATYANALSNQLAPQKGMVAAQHSLTFAANGWEPATAPNFGPLKVFYPGPGHTSDNITVGIDGTDIAFGGCLIKDSKAKSLGNLGDADTEHYAASARAFGAAFPKASMIVMSHSAPDSRAAITHTARMADKLR

SEQ ID NO: 89 - protein, 269 aa, artificial
  NDM-10
MELPNIMHPVAKLSTALAAALMLSGCMPGEISPTIDQQMETGDQRFGDLVFRQLAPNVWQHTSYLDMPSFGAVTSNGLIVRDGGRVLWDTAWTDDQTAQILNWIKQEINLPVALAVVTHAHQDKMGGMDALHAAGIATYANALSNQLAPQEGMVAAQHSLTFAANGWVEPATAPNFGPLKVFYPGPGHTSDNITVGIDRTDIAFGGCLIKDSKAKSLGNLGDADTEHYAASARAFGAAFPKASMIVMSHSAPDSRAAITHTARMADKLR

SEQ ID NO: 90 - protein, 268 aa, artificial
  NDM-11
MELPNIMHPVAKLSTALAAALMLSGCMPGEIRPTIGQQMETGDQRFGDLVFRQLAPNVWQHTSYLDMPGFGAVASNGLIVRDGGRVLVVDTAWTDDQTAQILNWIKQEINLPVALAWTHAHQDKMGGMDALHAAGIATYANALSNQLAPQEGLVAAQHSLTFAANGWEPATAPNFGPLKVFYPGPGHTSDNITVGIDGTDIAFGGCLIKDSKAKSLGNLDDADTEHYAASARAFGAAFPKASMIVMSHSAPDSRAAITHTARMADKLR

SEQ ID NO: 91 - protein, 268 aa, artificial; identical to SEQ ID NO: 90
  NDM-12

SEQ ID NO: 92 - protein, 268 aa, artificial
  NDM-13
MELPNIMHPVAKLSTALAAALMLSGCMPGEIRPTIGQQMETGDQRFGDLVFRQLAPNVWQHTSYLDMPGFGAVASNGLIVRDGGRVLVVDTAWTNDQTAQILNWIKQEINLPVALAWTHAHQDKMGGMDALHAAGIATYANALSNQLAPQEGLVAAQHSLTFAANGWEPATAPNFGPLKVFYPGPGHTSDNITVGIDGTDIAFGGCLIKDSKAKSLGNLGDADTEHYAASARAFGAAFPKASMIVMSHSAPDSRAAITHTARMADKLR

SEQ ID NO: 93 - protein, 260 aa, artificial
  P4A
EMKDDFAKLEEQFDAKLGIFALDTGTNRTVAYRPDERFAFASTIKALTVGVLLQQKSIEDLNQRITTRDDLVNYNPITEKHVDTGMTLKELADASLRYSDNAAQNLILKQIGGPESLKKELRKIGDEVTNPERFEPELNEVNPGETQDTSTARALVTSLRAFALEDKLPSEKRELLIDWMKRNTTGDALIRAGVPDGWEVGDKTGSGDYGTRNDIAIIWPPKGDPWLAVLSSRDKKDAKYDNKLIAEATKWMKALNMNGK

SEQ ID NO: 94 - protein, 299 aa, artificial; identical to SEQ ID NO: 65
  P4A + peptide signal

SEQ ID NO: 95 - protein, 263 aa, Escherichia coli
HPETLVKVKDAEDQLGARVGYIELDLNSGKILESFRPEERFPMVSTFKVLLCGAVLSRVDAGQEQLGRRIHYSQNDLVEYSPVTEKHLTDGMTVRELCSAAITMSDNTAANLLLTTIGGPKELTAFLHNMGDHVTRLDRWEPELNEAIPNDERDTTMPAAMATTLRKLLTGELLTLASRQQLIDWMEADKVAGPLLRSALPAGWFIADKSGAGERGSRGIIAALGPDGKPSRIVVIYTTGSQATMDERDRQIAEIGASLIKHW

SEQ ID NO: 96 - protein, 263 aa, Escherichia coli
QTSAVQQKLAALEKSSGGRLGVALIDTADNTQVLYRGDERFPMCSTSKVMAAAAVLKQSETQKQLLNQPVEIKPADLVNYNPIAEKHVNGTMTLAELSAAALQYSDNTAMNKLIAQLGGPGGVTAFARAIGDETFRLDRTEPTLNTAIPGDPRDTTTPRAMAQTLRQLTLGHALGETQRAQLVTWLKGNTTGAASIRAGLPTSWTAGDKTGSGGYGTTNDIAVIWPQGRAPLVLVTYFTQPQQNAESRRDVLASAARIIAEGL

SEQ ID NO: 97 - protein, 257 aa, Staphylococcus aureus
KELNDLEKKYNAHIGVYALDTKSGKEVKFNSDKRFAYASTSKAINSAILLEQVPYNKLNKKVHINKDDIVAYSPILEKYVGKDITLKALIEASMTYSDNTANNKIIKEIGGIKKVKQRLKELGDKVTNPVRYEIELNYYSPKSKKDTSTPAAFGKTLNKLIANGKLSKENKKFLLDLMLNNKSGDTLIKDGVPKDYKVADKSGQAITYASRNDVAFVYPKGQSEPIVLVIFTNKDNKSDKPNDKLISETAKSVMKEF

SEQ ID NO: 98 - protein, 199 aa, Escherichia coli
MSNAKTKLGITKYSIVTNSNDSVTLRLMTEHDLAMLYEWLNRSHIVEWWGGEEARPTLADVQEQYLPSVLAQESVTPYIAMLNGEPIGYAQSYVALGSGDGRWEEETDPGVRGIDQLLANASQLGKGLGTKLVRALVELLFNDPEVTKIQTDPSPSNLRAIRCYEKAGFERQGTVTTPYGPAVYMVQTRQAFERTRSDA

SEQ ID NO: 99 - protein, 419 aa, Escherichia coli
MRFEEWVKDKHIPFKLNHPDDNYDDFKPLRKIIGDTRVVALGENSHFIKEFFLLRHTLLRFFIEDLGFTTFAFEFGFAEGQIINNWIHGQGTDDEIGRFLKHFYYPEELKTTFLWLREYNKAAKEKITFLGIDIPRNGGSYLPNMEIVHDFFRTADKEALHIIDDAFNIAKKIDYFSTSQAALNLHELTDSEKCRLTSQLARVKVRLEAMAPIHIEKYGIDKYETILHYANGMIYLDYNIQAMSGFISGGGMQGDMGAKDKYMADSVLWHLKNPQSEQKVIVVAHNAHIQKTPILYDGFLSCLPMGQRLKNAIGDDYMSLGITSYSGHTAALYPEVDTKYGFRVDNFQLQEPNEGSVEKAISGCGVTNSFVFFRNIPEDLQSIPNMIRFDSIYMKAELEKAFDGIFQIEKSSVSEVVYE

SEQ ID NO: 100 - protein, 388 aa, Bacteroides fragilis
MTMRIDTDKQMNLLSDKNVAIIGGGPVGLTMAKLLQQNGIDVSVYERDNDREARIFGGTLDLHKGSGQEAMKKAGLLQTYYDLALPMGVNIADKKGNILSTKNVKPENRFDNPEINRNDLRAILLNSLENDTVIWDRKLVMLEPGKKKWTLTFENKPSETADLVILANGGMSKVRKFVTDTEVEETGTFNIQADIHQPEINCPGFFQLCNGNRLMASHQGNLLFANPNNNGALHFGISFKTPDEWKNQTQVDFQNRNSVVDFLLKEFSDWDERYKELIHTTLSFVGLATRIFPLEKPWKSKRPLPITMIGDAAHLMPPFAGQGVNSGLVDALILSDNLADGKFNSIEEAVKNYEQQMFMYGKEAQEESTQNEIEMFKPDFTFQQLLNV

SEQ ID NO: 101 - protein, 267 aa, Enterococcus faecium
MLKQKELIANVKNLTESDERITACMMYGSFTKGEGDQYSDIEFYIFLKHSITSNFDSSNWLFDVAPYLMLYKNEYGTEVVIFDNLIRGEFHFLSEKDMNIIPSFKDSGYIPDTKAMLIYDETGQLENYLSEISGARPNRLTEENANFLLCNFSNLWLMGINVLKRGEYARSLELLSQLQKNTLQLIRMAEKNADNWLNMSKNLEKEISLENYKKFAKTTARLDKVELFEAYKNSLLLVMDLQSHLIEQYNLKVTHDILERLLNYISE

SEQ ID NO: 102 - protein, 532 aa, artificial
  hybrid protein TEM36-GGGGGG-CTXM16
HPETLVKVKDAEDQLGARVGYIELDLNSGKILESFRPEERFPMVSTFKVLLCGAVLSRVDAGQEQLGRRIHYSQNDLVEYSPVTEKHLTDGMTVRELCSAAITMSDNTAANLLLTTIGGPKELTAFLHNMGDHVTRLDRWEPELNEAIPNDERDTTMPAAMATTLRKLLTGELLTLASRQQLIDWMEADKVAGPLLRSALPAGWFIADKSGAGERGSRGIIAALGPDGKPSRIVVIYTTGSQATMDERDRQIAEIGASLIKHWGGGGGGQTSAVQQKLAALEKSSGGRLGVALIDTADNTQVLYRGDERFPMCSTSKVMAAAAVLKQSETQKQLLNQPVEIKPADLVNYNPIAEKHVNGTMTLAELSAAALQYSDNTAMNKLIAQLGGPGGVTAFARAIGDETFRLDRTEPTLNTAIPGDPRDTTTPRAMAQTLRQLTLGHALGETQRAQLVTWLKGNTTGAASIRAGLPTSWTAGDKTGSGGYGTTNDIAVIWPQGRAPLVLVTYFTQPQQNAESRRDVLASAARIIAEGL

SEQ ID NO: 103 - protein, 532 aa, artificial
  fusion CTXM16-6G-TEM36
QTSAVQQKLAALEKSSGGRLGVALIDTADNTQVLYRGDERFPMCSTSKVMAAAAVLKQSETQKQLLNQPVEIKPADLVNYNPIAEKHVNGTMTLAELSAAALQYSDNTAMNKLIAQLGGPGGVTAFARAIGDETFRLDRTEPTLNTAIPGDPRDTTTPRAMAQTLRQLTLGHALGETQRAQLVTWLKGNTTGAASIRAGLPTSWTAGDKTGSGGYGTTNDIAVIWPQGRAPLVLVTYFTQPQQNAESRRDVLASAARIIAEGLGGGGGGHPETLVKVKDAEDQLGARVGYIELDLNSGKILESFRPEERFPMVSTFKVLLCGAVLSRVDAGQEQLGRRIHYSQNDLVEYSPVTEKHLTDGMTVRELCSAAITMSDNTAANLLLTTIGGPKELTAFLHNMGDHVTRLDRWEPELNEAIPNDERDTTMPAAMATTLRKLLTGELLTLASRQQLIDWMEADKVAGPLLRSALPAGWFIADKSGAGERGSRGIIAALGPDGKPSRIVVIYTTGSQATMDERDRQIAEIGASLIKHW

SEQ ID NO: 104 - protein, 537 aa, artificial
  fusion CTXM16-6G-TEM36
HPETLVKVKDAEDQLGARVGYIELDLNSGKILESFRPEERFPMVSTFKVLLCGAVLSRVDAGQEQLGRRIHYSQNDLVEYSPVTEKHLTDGMTVRELCSAAITMSDNTAANLLLTTIGGPKELTAFLHNMGDHVTRLDRWEPELNEAIPNDERDTTMPAAMATTLRKLLTGELLTLASRQQLIDWMEADKVAGPLLRSALPAGWFIADKSGAGERGSRGIIAALGPDGKPSRIVVIYTTGSQATMDERDRQIAEIGASLIKHWGEAAAKEAAAKQTSAVQQKLAALEKSSGGRLGVALIDTADNTQVLYRGDERFPMCSTSKVMAAAAVLKQSETQKQLLNQPVEIKPADLVNYNPIAEKHVNGTMTLAELSAAALQYSDNTAMNKLIAQLGGPGGVTAFARAIGDETFRLDRTEPTLNTAIPGDPRDTTTPRAMAQTLRQLTLGHALGETQRAQLVTWLKGNTTGAASIRAGLPTSWTAGDKTGSGGYGTTNDIAVIWPQGRAPLVLVTYFTQPQQNAESRRDVLASAARIIAEGL

SEQ ID NO: 105 - DNA, 116 bp, artificial
  modified intron "INT1"
gtatgtatataagaatttttcctcccactttattgtttctaaaagttcaatgaagtaaagtctaaattggccttattactaactaataggtatcttataatcacctaataaaatag

SEQ ID NO: 106 - protein, 266 aa, artificial
  VIM 2 WT, full length
MFKLLSKLLVYLTASIMAIASPLAFSVDSSGEYPTVSEIPVGEVRLYQIADGVWSHIATQSFDGAVYPSNGLIVRDGDELLLIDTAWGAKNTAALLAEIEKQIGLPVTRAVSTHFHDDRVGGVDVLRAAGVATYASPSTRRLAEVEGNEIPTHSLEGLSSSGDAVRFGPVELFYPGAAHSTDNLVVYVPSASVLYGGCAIYELSRTSAGNVADADLAEWPTSIERIQQHYPEAQFVIPGHGLPGGLDLLKHTTNVVKAHTNRSVVE

SEQ ID NO: 107 - DNA, 801 bp, artificial
  Nucleic sequence encoding full length VIM-2 WT
atgttcaaacttttgagtaagttattggtctatttgaccgcgtctatcatggctattgcgagtccgctcgctttttccgtagattctagcggtgagtatccgacagtcagcgaaattccggtcggggaggtccggctttaccagattgccgatggtgtttggtcgcatatcgcaacgcagtcgtttgatggcgcagtctacccgtccaatggtctcattgtccgtgatggtgatgagttgcttttgattgatacagcgtggggtgcgaaaaacacagcggcacttctcgcggagattgagaagcaaattggacttcctgtaacgcgtgcagtctccacgcactttcatgacgaccgcgtcggcggcgttgatgtccttcgggcggctggggtggcaacgtacgcatcaccgtcgacacgccggctagccgaggtagaggggaacgagattcccacgcactctctagaaggactctcatcgagcggggacgcagtgcgcttcggtccagtagaactcttctatcctggtgctgcgcattcgaccgacaacttagttgtgtacgtcccgtctgcgagtgtgctctatggtggttgtgcgatttatgagttgtcacgcacgtctgcggggaacgtggccgatgccgatctggctgaatggcccacctccattgagcggattcaacaacactacccggaagcacagttcgtcattccggggcacggcctgccgggcggtctagacttgctcaagcacacaacgaatgttgtaaaagcgcacacaaatcgctcagtcgttgagtag

SEQ ID NO: 108 - protein, 264 aa, artificial
  sequence P3A variants "long version"
  misc_feature (245)..(245): Xaa can be any naturally occurring amino acid
TEMKDDFAKLEEQFDAKLGIFALDTGTNRTVAYRPDERFAFASTIKALTVGVLLQQKSIEDLNQRITYTRDDLVNYNPITEKHVDTGMTLKELADASLRYSDNAAQNLILKQIGGPESLKKELRKIGDEVTNPERFEPELNEVNPGETQDTSTARALVTSLRAFALEDKLPSEKRELLIDWMKRNTTGDALIRAGVPDGWEVADKTGAASYGTRNDIAIIWPPKGDPVVLAVLSSRDKKDAKYDXKLIAEATKVVMKALNMNGK

SEQ ID NO: 109 - DNA, 795 bp, artificial
  sequence encoding P3A version " long version "
  misc_feature (736)..(738): n is a, c, g, or t
atgactgagatgaaagatgattttgcgaagctggaagaacagtttgacgcaaaattgggcattttcgcgttggacacgggtacgaatcgtacggttgcctaccgtccggacgagcgcttcgccttcgcgagcacgatcaaagccctgaccgtcggcgtgctgctccagcaaaagagcatcgaggacctgaaccagcgcattacctacacccgtgatgatctggtgaactataatccgatcaccgagaaacacgttgataccggtatgaccctgaaagaactggcagatgcaagcctgcgctacagcgataacgcggctcagaatctgattctgaagcaaatcggtggtccggagagcttgaagaaagaactgcgtaaaatcggcgatgaagtcactaatccggagcgttttgagccggagctgaacgaagtgaatccgggtgaaacgcaagacacgagcaccgcgcgtgcgcttgtcacctccctgcgcgctttcgcactggaagataagctgccgtcggagaaacgcgagctgctgatcgactggatgaagcgcaatacgaccggcgacgcgctgattcgtgcgggcgttccggacggttgggaagtggctgacaagaccggtgcggcgagctacggcacccgtaacgatatcgcgatcatttggccacctaaaggtgacccggtcgtgctggccgtactgagcagccgtgacaagaaagacgcaaagtatgatnnnaagctgattgcagaggcgaccaaagttgttatgaaggcactgaacatgaatggtaag

SEQ ID NO: 110 - DNA, 270 bp, artificial
  alpha-factor signal (nucleic sequence)- variant
atgagatttccttcaatttttactgctgttttattcgcagcatcctccgcattagctgctccagtcaacactacaacagaagatgaaacggcacaaattccggctgaagctgtcatcggttactcagatttagaaggggatttcgatgttgctgttttgccattttccaacagcacaaataacgggttattgtttataaatactactattgccagcattgctgctaaagaagaaggggtatctctcgagaaaagagaggctgaagctctg

SEQ ID NO: 111 - protein, 90 aa, artificial
  alpha factor signal (protein sequence)- variant
MRFPSIFTAVLFAASSALAAPVNTTTEDETAQIPAEAVIGYSDLEGDFDVAVLPFSNSTNNGLLFINTTIASIAAKEEGVSLEKREAEAL

SEQ ID NO: 112 - DNA, 60 bp, artificial
  K1 signal peptide of K. lactis (nucleic sequence) - variant
atgaatatattttacatatttttgtttttgctgtcattcgttcaaggtacccggggatcc

SEQ ID NO: 113 - protein, 20 aa, artificial
  K1 signal peptide of K. lactis (protein sequence)- variant
MNIFYIFLFLLSFVQGTRGS

SEQ ID NO: 114 - DNA, 846 bp, artificial
  modified version of the beta lactamase BL gene
atgaatatattttacatatttttgtttttgctgtcattcgttcaaggtacccggggatccaaggacgacttcgctaagttggaagaacaattcgacgctaagttgggtatcttcgctttggacactggtactaacagaactgttgcttacagaccagacgaaagattcgctttcgcttctactatcaaggctttgactgttggtgttttgttgcaacaaaagtctatcgaagacttgaaccaaagaatcacttacactagagacgacttggttaactacaacccaatcactgaaaagcacgttgacactggtatgactttgaaggaattggctgacgcttctttgagatactctgacaacgctgctcaaaacttgatcttgaagcaaatcggtggtccagaatctttgaagaaggaattgagaaagatcggtgacgaagttactaacccagaaagattcgaaccagaattgaacgaagttaacccaggtgaaactcaagacacttctactgctagagctttggttacttctttgagagctttcgctttggaagacaagttgccatctgaaaagagagaattgttgatcgactggatgaagagaaacactactggtgacgctttgatcagagctggtgttccagacggttgggaagttgctgacaagactggtgctgcttcttacggtactaaaaacgacatcgctatcatctggccaccaaagggtgacccagttgttttggctgttttgtcttctagagacaagaaggacgctaagtacgacaacaagttgatcgctgaagctactaaggttgttatgaaggctttgaacatgaacggtaagtaa